European Patent Application EP 4 393 959 A1, published July 3, 2024. Title: Human transferrin receptor binding peptide - antibody conjugates. Applicant: PeptiDream INC. Application JP. The sequence listing filed with the application follows.

SEQUENCE LISTING (161 sequences)

SEQ ID NO: 1 - protein, 15 aa, synthetic construct
  REGION 1..15: note = Synthesized polypeptide
  MOD_RES 14: note = METHYLATION
AVFVWNYYIIRRYYC

SEQ ID NO: 2 - protein, 15 aa, synthetic construct
  REGION 1..15: note = Synthesized polypeptide
  MOD_RES 14: note = METHYLATION
AVFVWNYYIIRRYYC

SEQ ID NO: 3 - protein, 15 aa, synthetic construct
  REGION 1..15: note = Synthesized polypeptide
  MOD_RES 14: note = METHYLATION
AVFVWNYYIIARYYC

SEQ ID NO: 4 - protein, 15 aa, synthetic construct
  REGION 1..15: note = Synthesized polypeptide
  MOD_RES 14: note = METHYLATION
AVFVWNYYIIRRYYC

SEQ ID NO: 5 - protein, 15 aa, synthetic construct
  REGION 1..15: note = Synthesized polypeptide
  MOD_RES 14: note = METHYLATION
AVFVWNYYIIARYYC

SEQ ID NO: 6 - protein, 15 aa, synthetic construct
  REGION 1..15: note = Synthesized polypeptide
  MOD_RES 14: note = METHYLATION
AVFVWNYYIIRRYYC

SEQ ID NO: 7 - protein, 15 aa, synthetic construct
  REGION 1..15: note = Synthesized polypeptide
  MOD_RES 14: note = METHYLATION
AVFVWNYYIIRRYYC

SEQ ID NO: 8 - protein, 15 aa, synthetic construct
  REGION 1..15: note = Synthesized polypeptide
  MOD_RES 14: note = METHYLATION
AVFVWNYYIIARYYC

SEQ ID NO: 9 - protein, 15 aa, synthetic construct
  REGION 1..15: note = Synthesized polypeptide
  MOD_RES 14: note = METHYLATION
AVFVWNYYIIAEYYC

SEQ ID NO: 10 - protein, 15 aa, synthetic construct
  REGION 1..15: note = Synthesized polypeptide
  MOD_RES 14: note = METHYLATION
AVFVWNYYIIEEYYC

SEQ ID NO: 11 - protein, 15 aa, synthetic construct
  REGION 1..15: note = Synthesized polypeptide
  MOD_RES 14: note = METHYLATION
AVFVWNYYIIRRYYC

SEQ ID NO: 12 - protein, 15 aa, synthetic construct
  REGION 1..15: note = Synthesized polypeptide
  MOD_RES 14: note = METHYLATION
AVFVWNYYIIRRYYC

SEQ ID NO: 13 - protein, 15 aa, synthetic construct
  REGION 1..15: note = Synthesized polypeptide
  MOD_RES 14: note = METHYLATION
AVFVWNYYIIRRYYC

SEQ ID NO: 14 - protein, 12 aa, synthetic construct
  REGION 1..12: note = Synthesized polypeptide
AVFVWNYYIISC

SEQ ID NO: 15 - protein, 15 aa, synthetic construct
  REGION 1..15: note = Synthesized polypeptide
  MOD_RES 3: note = METHYLATION
  MOD_RES 14: note = METHYLATION
AVFVWNYYIIRRYYC

SEQ ID NO: 16 - protein, 12 aa, synthetic construct
  REGION 1..12: note = Synthesized polypeptide
AVFVWNYYIISC

SEQ ID NO: 17 - protein, 12 aa, synthetic construct
  REGION 1..12: note = Synthesized polypeptide
AVFVWNYYIISC

SEQ ID NO: 18 - protein, 15 aa, synthetic construct
  REGION 1..15: note = Synthesized polypeptide
  MOD_RES 3: note = METHYLATION
  MOD_RES 14: note = METHYLATION
AVFVWNYYIIRRYYC

SEQ ID NO: 19 - protein, 15 aa, synthetic construct
  REGION 1..15: note = Synthesized polypeptide
  MOD_RES 14: note = METHYLATION
AVFVWNYYIIRRYYC

SEQ ID NO: 20 - protein, 15 aa, synthetic construct
  REGION 1..15: note = Synthesized polypeptide
  MOD_RES 3: note = METHYLATION
  MOD_RES 14: note = METHYLATION
AVFVWNYYIARRYYC

SEQ ID NO: 21 - protein, 15 aa, synthetic construct
  REGION 1..15: note = Synthesized polypeptide
  MOD_RES 3: note = METHYLATION
  MOD_RES 14: note = METHYLATION
AVFVWAYYIIRRYYC

SEQ ID NO: 22 - protein, 15 aa, synthetic construct
  REGION 1..15: note = Synthesized polypeptide
  SITE 3: note = MISC_FEATURE - Xaa is MeF3C
  MOD_RES 5: note = METHYLATION
  SITE 8: note = MISC_FEATURE - Xaa is F4OMe
  SITE 12: note = MISC_FEATURE - Xaa is dr
  MOD_RES 14: note = METHYLATION
AVXVWNYXIIRXFYC

SEQ ID NO: 23 - protein, 15 aa, synthetic construct
  REGION 1..15: note = Synthesized polypeptide
  SITE 2: note = MISC_FEATURE - Xaa is Hgl
  SITE 3: note = MISC_FEATURE - Xaa is MeF3C
  MOD_RES 5: note = METHYLATION
  SITE 11: note = MISC_FEATURE - Xaa is Hly
  MOD_RES 14: note = METHYLATION
AXXVWNYYIIXRYYC

SEQ ID NO: 24 - protein, 15 aa, synthetic construct
  REGION 1..15: note = Synthesized polypeptide
  MOD_RES 3: note = METHYLATION
  MOD_RES 14: note = METHYLATION
AVFVWNYYIIRRYYC

SEQ ID NO: 25 - protein, 15 aa, synthetic construct
  REGION 1..15: note = Synthesized polypeptide
  MOD_RES 3: note = METHYLATION
  MOD_RES 14: note = METHYLATION
AVFVWNYYIIRRYYC

SEQ ID NO: 26 - protein, 15 aa, synthetic construct
  REGION 1..15: note = Synthesized polypeptide
  MOD_RES 3: note = METHYLATION
  MOD_RES 14: note = METHYLATION
AVFVWNYYIIRRYYC

SEQ ID NO: 27 - protein, 15 aa, synthetic construct
  REGION 1..15: note = Synthesized polypeptide
  MOD_RES 3: note = METHYLATION
  MOD_RES 14: note = METHYLATION
AVFVWNYYIIRRYYC

SEQ ID NO: 28 - protein, 15 aa, synthetic construct
  REGION 1..15: note = Synthesized polypeptide
  MOD_RES 3: note = METHYLATION
  MOD_RES 14: note = METHYLATION
AVFVWNYYIIRRYYC

SEQ ID NO: 29 - protein, 15 aa, synthetic construct
  REGION 1..15: note = Synthesized polypeptide
  MOD_RES 3: note = METHYLATION
  MOD_RES 14: note = METHYLATION
AVFVWNYYIIRRYYC

SEQ ID NO: 30 - protein, 15 aa, synthetic construct
  REGION 1..15: note = Synthesized polypeptide
  MOD_RES 3: note = METHYLATION
  MOD_RES 14: note = METHYLATION
AVFVWNYYIIRRYYC

SEQ ID NO: 31 - protein, 15 aa, synthetic construct
  REGION 1..15: note = Synthesized polypeptide
  MOD_RES 3: note = METHYLATION
  MOD_RES 14: note = METHYLATION
AVFVWNYYIIRRYYC

SEQ ID NO: 32 - protein, 15 aa, synthetic construct
  REGION 1..15: note = Synthesized polypeptide
  MOD_RES 3: note = METHYLATION
  MOD_RES 14: note = METHYLATION
AVFVWNYYIIRRYYC

SEQ ID NO: 33 - protein, 15 aa, synthetic construct
  REGION 1..15: note = Synthesized polypeptide
  MOD_RES 14: note = METHYLATION
AVFVWNYYIIRRYYC

SEQ ID NO: 34 - protein, 15 aa, synthetic construct
  REGION 1..15: note = Synthesized polypeptide
  MOD_RES 3: note = METHYLATION
  MOD_RES 14: note = METHYLATION
AVFVWNYYIIRRYYC

SEQ ID NO: 35 - protein, 15 aa, synthetic construct
  REGION 1..15: note = Synthesized polypeptide
  MOD_RES 3: note = METHYLATION
  MOD_RES 14: note = METHYLATION
AVFVWNYYIIRRYYC

SEQ ID NO: 36 - protein, 15 aa, synthetic construct
  REGION 1..15: note = Synthesized polypeptide
  MOD_RES 3: note = METHYLATION
  MOD_RES 14: note = METHYLATION
AVFVWNYYIIRRYYC

SEQ ID NO: 37 - protein, 15 aa, synthetic construct
  REGION 1..15: note = Synthesized polypeptide
  MOD_RES 3: note = METHYLATION
  MOD_RES 14: note = METHYLATION
AVFVWNYYIIRRYYC

SEQ ID NO: 38 - protein, 15 aa, synthetic construct
  REGION 1..15: note = Synthesized polypeptide
  MOD_RES 5: note = METHYLATION
  MOD_RES 14: note = METHYLATION
AVFVWNYYIIRRYYC

SEQ ID NO: 39 - protein, 15 aa, synthetic construct
  REGION 1..15: note = Synthesized polypeptide
  MOD_RES 5: note = METHYLATION
  MOD_RES 14: note = METHYLATION
AVFVWNYYIIRRYYC

SEQ ID NO: 40 - protein, 15 aa, synthetic construct
  REGION 1..15: note = Synthesized polypeptide
  MOD_RES 5: note = METHYLATION
  MOD_RES 14: note = METHYLATION
AVFVWNYYIIRRYYC

SEQ ID NO: 41 - protein, 15 aa, synthetic construct
  REGION 1..15: note = Synthesized polypeptide
  MOD_RES 5: note = METHYLATION
  MOD_RES 14: note = METHYLATION
AVFVWNYYIIRRYYC

SEQ ID NO: 42 - protein, 15 aa, synthetic construct
  REGION 1..15: note = Synthesized polypeptide
  MOD_RES 3: note = METHYLATION
  MOD_RES 5: note = METHYLATION
  MOD_RES 14: note = METHYLATION
AVFVWNYYIIRRYYC

SEQ ID NO: 43 - protein, 15 aa, synthetic construct
  REGION 1..15: note = Synthesized polypeptide
  MOD_RES 3: note = METHYLATION
  MOD_RES 5: note = METHYLATION
  MOD_RES 14: note = METHYLATION
AVFVWNYYIIRRYYC

SEQ ID NO: 44 - protein, 15 aa, synthetic construct
  REGION 1..15: note = Synthesized polypeptide
  MOD_RES 3: note = METHYLATION
  MOD_RES 5: note = METHYLATION
  MOD_RES 14: note = METHYLATION
AVFVWNYYIIRRYYC

SEQ ID NO: 45 - protein, 15 aa, synthetic construct
  REGION 1..15: note = Synthesized polypeptide
  MOD_RES 3: note = METHYLATION
  MOD_RES 5: note = METHYLATION
  MOD_RES 14: note = METHYLATION
AVFVWNYYIIRRYYC

SEQ ID NO: 46 - protein, 15 aa, synthetic construct
  REGION 1..15: note = Synthesized polypeptide
  MOD_RES 14: note = METHYLATION
AVFVWNYYIIKRYYC

SEQ ID NO: 47 - protein, 15 aa, synthetic construct
  REGION 1..15: note = Synthesized polypeptide
  MOD_RES 14: note = METHYLATION
AVFVWNYYIIKRYYC

SEQ ID NO: 48 - protein, 15 aa, synthetic construct
  REGION 1..15: note = Synthesized polypeptide
  MOD_RES 14: note = METHYLATION
AVFVWNYYIIKRYYC

SEQ ID NO: 49 - protein, 15 aa, synthetic construct
  REGION 1..15: note = Synthesized polypeptide
  MOD_RES 14: note = METHYLATION
AVFVWNYYIIKRYYC

SEQ ID NO: 50 - protein, 15 aa, synthetic construct
  REGION 1..15: note = Synthesized polypeptide
  MOD_RES 3: note = METHYLATION
  MOD_RES 14: note = METHYLATION
AVFVWNYYIIKRYYC

SEQ ID NO: 51 - protein, 15 aa, synthetic construct
  REGION 1..15: note = Synthesized polypeptide
  MOD_RES 3: note = METHYLATION
  MOD_RES 14: note = METHYLATION
AVFVWNYYIIKRYYC

SEQ ID NO: 52 - protein, 15 aa, synthetic construct
  REGION 1..15: note = Synthesized polypeptide
  MOD_RES 3: note = METHYLATION
  MOD_RES 14: note = METHYLATION
AVFVWNYYIIKRYYC

SEQ ID NO: 53 - protein, 15 aa, synthetic construct
  REGION 1..15: note = Synthesized polypeptide
  MOD_RES 3: note = METHYLATION
  MOD_RES 14: note = METHYLATION
AVFVWNYYIIKRYYC

SEQ ID NO: 54 - protein, 15 aa, synthetic construct
  REGION 1..15: note = Synthesized polypeptide
  MOD_RES 3: note = METHYLATION
  MOD_RES 5: note = METHYLATION
  MOD_RES 14: note = METHYLATION
AVFVWNYYIIKRYYC

SEQ ID NO: 55 - protein, 15 aa, synthetic construct
  REGION 1..15: note = Synthesized polypeptide
  MOD_RES 3: note = METHYLATION
  MOD_RES 5: note = METHYLATION
  MOD_RES 14: note = METHYLATION
AVFVWNYYIIKRYYC

SEQ ID NO: 56 - protein, 15 aa, synthetic construct
  REGION 1..15: note = Synthesized polypeptide
  MOD_RES 3: note = METHYLATION
  MOD_RES 5: note = METHYLATION
  MOD_RES 14: note = METHYLATION
AVFVWNYYIIKRYYC

SEQ ID NO: 57 - protein, 15 aa, synthetic construct
  REGION 1..15: note = Synthesized polypeptide
  MOD_RES 3: note = METHYLATION
  MOD_RES 5: note = METHYLATION
  MOD_RES 14: note = METHYLATION
AVFVWNYYIIKRYYC

SEQ ID NO: 58 - protein, 15 aa, synthetic construct
  REGION 1..15: note = Synthesized polypeptide
  MOD_RES 3: note = METHYLATION
  MOD_RES 14: note = METHYLATION
AVFVWNYYIIRRYYC

SEQ ID NO: 59 - protein, 15 aa, synthetic construct
  REGION 1..15: note = Synthesized polypeptide
  MOD_RES 3: note = METHYLATION
  MOD_RES 14: note = METHYLATION
AVFVWNYYIIRRYYC

SEQ ID NO: 60 - protein, 15 aa, synthetic construct
  REGION 1..15: note = Synthesized polypeptide
  MOD_RES 3: note = METHYLATION
  MOD_RES 14: note = METHYLATION
AVFVWNYYIIRRYYC

SEQ ID NO: 61 - protein, 15 aa, synthetic construct
  REGION 1..15: note = Synthesized polypeptide
  MOD_RES 3: note = METHYLATION
  MOD_RES 14: note = METHYLATION
AVFVWNYYIIRRYYC

SEQ ID NO: 62 - protein, 15 aa, synthetic construct
  REGION 1..15: note = Synthesized polypeptide
  MOD_RES 3: note = METHYLATION
  MOD_RES 14: note = METHYLATION
AVFVWNYYIIRRYYC

SEQ ID NO: 63 - protein, 15 aa, synthetic construct
  REGION 1..15: note = Synthesized polypeptide
  MOD_RES 3: note = METHYLATION
  MOD_RES 14: note = METHYLATION
AVFVWNYYIIRRYYC

SEQ ID NO: 64 - protein, 15 aa, synthetic construct
  REGION 1..15: note = Synthesized polypeptide
  MOD_RES 3: note = METHYLATION
  MOD_RES 14: note = METHYLATION
AVFVWNYYIIRRYYC

SEQ ID NO: 65 - protein, 15 aa, synthetic construct
  REGION 1..15: note = Synthesized polypeptide
  MOD_RES 3: note = METHYLATION
  MOD_RES 14: note = METHYLATION
AVFVWNYYIIRRYYC

SEQ ID NO: 66 - protein, 15 aa, synthetic construct
  REGION 1..15: note = Synthesized polypeptide
  MOD_RES 3: note = METHYLATION
  MOD_RES 14: note = METHYLATION
AVFVWNYYIIRRYYC

SEQ ID NO: 67 - protein, 15 aa, synthetic construct
  REGION 1..15: note = Synthesized polypeptide
  MOD_RES 3: note = METHYLATION
  MOD_RES 14: note = METHYLATION
AVFVWNYYIIRRYYC

SEQ ID NO: 68 - protein, 15 aa, synthetic construct
  REGION 1..15: note = Synthesized polypeptide
  MOD_RES 3: note = METHYLATION
  MOD_RES 14: note = METHYLATION
AVFVWNYYIIRRYYC

SEQ ID NO: 69 - protein, 15 aa, synthetic construct
  REGION 1..15: note = Synthesized polypeptide
  MOD_RES 3: note = METHYLATION
  MOD_RES 14: note = METHYLATION
AVFVWNYYIIRRYYC

SEQ ID NO: 70 - protein, 15 aa, synthetic construct
  REGION 1..15: note = Synthesized polypeptide
  MOD_RES 3: note = METHYLATION
  MOD_RES 14: note = METHYLATION
AVFVWNYYIIRRYYC

SEQ ID NO: 71 - protein, 15 aa, synthetic construct
  REGION 1..15: note = Synthesized polypeptide
  MOD_RES 3: note = METHYLATION
  MOD_RES 14: note = METHYLATION
AVFVWNYYIIRRYYC

SEQ ID NO: 72 - protein, 15 aa, synthetic construct
  REGION 1..15: note = Synthesized polypeptide
  MOD_RES 5: note = METHYLATION
  MOD_RES 14: note = METHYLATION
AVFVWNYYIIRRYYC

SEQ ID NO: 73 - protein, 15 aa, synthetic construct
  REGION 1..15: note = Synthesized polypeptide
  MOD_RES 5: note = METHYLATION
  MOD_RES 14: note = METHYLATION
AVFVWNYYIIRRYYC

SEQ ID NO: 74 - protein, 15 aa, synthetic construct
  REGION 1..15: note = Synthesized polypeptide
  MOD_RES 5: note = METHYLATION
  MOD_RES 14: note = METHYLATION
AVFVWNYYIIRRYYC

SEQ ID NO: 75 - protein, 15 aa, synthetic construct
  REGION 1..15: note = Synthesized polypeptide
  MOD_RES 5: note = METHYLATION
  MOD_RES 14: note = METHYLATION
AVFVWNYYIIRRYYC

SEQ ID NO: 76 - protein, 15 aa, synthetic construct
  REGION 1..15: note = Synthesized polypeptide
  MOD_RES 5: note = METHYLATION
  MOD_RES 14: note = METHYLATION
AVFVWNYYIIRRYYC

SEQ ID NO: 77 - protein, 15 aa, synthetic construct
  REGION 1..15: note = Synthesized polypeptide
  MOD_RES 3: note = METHYLATION
  MOD_RES 5: note = METHYLATION
  MOD_RES 14: note = METHYLATION
AVFVWNYYIIRRYYC

SEQ ID NO: 78 - protein, 15 aa, synthetic construct
  REGION 1..15: note = Synthesized polypeptide
  MOD_RES 3: note = METHYLATION
  MOD_RES 5: note = METHYLATION
  MOD_RES 14: note = METHYLATION
AVFVWNYYIIRRYYC

SEQ ID NO: 79 - protein, 15 aa, synthetic construct
  REGION 1..15: note = Synthesized polypeptide
  MOD_RES 3: note = METHYLATION
  MOD_RES 5: note = METHYLATION
  MOD_RES 14: note = METHYLATION
AVFVWNYYIIRRYYC

SEQ ID NO: 80 - protein, 15 aa, synthetic construct
  REGION 1..15: note = Synthesized polypeptide
  MOD_RES 3: note = METHYLATION
  MOD_RES 5: note = METHYLATION
  MOD_RES 14: note = METHYLATION
AVFVWNYYIIRRYYC

SEQ ID NO: 81 - protein, 15 aa, synthetic construct
  REGION 1..15: note = Synthesized polypeptide
  MOD_RES 3: note = METHYLATION
  MOD_RES 5: note = METHYLATION
  MOD_RES 14: note = METHYLATION
AVFVWNYYIIRRYYC

SEQ ID NO: 82 - protein, 15 aa, synthetic construct
  REGION 1..15: note = Synthesized polypeptide
  MOD_RES 3: note = METHYLATION
  MOD_RES 14: note = METHYLATION
AVFVWNYYIIRRYYC

SEQ ID NO: 83 - protein, 15 aa, synthetic construct
  REGION 1..15: note = Synthesized polypeptide
  MOD_RES 5: note = METHYLATION
  MOD_RES 14: note = METHYLATION
AVFVWNYYIIRRYYC

SEQ ID NO: 84 - protein, 15 aa, synthetic construct
  REGION 1..15: note = Synthesized polypeptide
  MOD_RES 5: note = METHYLATION
  MOD_RES 14: note = METHYLATION
AVFVWNYYIIRRYYC

SEQ ID NO: 85 - protein, 15 aa, synthetic construct
  REGION 1..15: note = Synthesized polypeptide
  MOD_RES 3: note = METHYLATION
  MOD_RES 5: note = METHYLATION
  MOD_RES 14: note = METHYLATION
AVFVWNYYIIRRYYC

SEQ ID NO: 86 - protein, 15 aa, synthetic construct
  REGION 1..15: note = Synthesized polypeptide
  MOD_RES 3: note = METHYLATION
  MOD_RES 5: note = METHYLATION
  MOD_RES 14: note = METHYLATION
AVFVWNYYIIRRYYC

SEQ ID NO: 87 - protein, 12 aa, synthetic construct
  REGION 1..12: note = Synthesized polypeptide
AVFVWNYYIISC

SEQ ID NO: 88 - protein, 12 aa, synthetic construct
  REGION 1..12: note = Synthesized polypeptide
AVFVWNYYIISC

SEQ ID NO: 89 - protein, 12 aa, synthetic construct
  REGION 1..12: note = Synthesized polypeptide
AVFVWNYYIISC

SEQ ID NO: 90 - protein, 15 aa, synthetic construct
  REGION 1..15: note = Synthesized polypeptide
  SITE 1: note = MISC_FEATURE - Xaa is Abu
  MOD_RES 3: note = METHYLATION
  MOD_RES 14: note = METHYLATION
XVFVWNYYIIRRYYC

SEQ ID NO: 91 - protein, 15 aa, synthetic construct
  REGION 1..15: note = Synthesized polypeptide
  SITE 1: note = MISC_FEATURE - Xaa is Abu
  MOD_RES 3: note = METHYLATION
  MOD_RES 14: note = METHYLATION
XVFVWNYYIIRRYYC

SEQ ID NO: 92 - protein, 15 aa, synthetic construct
  REGION 1..15: note = Synthesized polypeptide
  SITE 1: note = MISC_FEATURE - Xaa is Abu
  MOD_RES 3: note = METHYLATION
  MOD_RES 14: note = METHYLATION
XVFVWNYYIIRRYYC

SEQ ID NO: 93 - protein, 15 aa, synthetic construct
  REGION 1..15: note = Synthesized polypeptide
  MOD_RES 3: note = METHYLATION
  SITE 8: note = MISC_FEATURE - Xaa is Ahp
  MOD_RES 14: note = METHYLATION
AVFVWNYXIIRRYYC

SEQ ID NO: 94 - protein, 15 aa, synthetic construct
  REGION 1..15: note = Synthesized polypeptide
  MOD_RES 3: note = METHYLATION
  SITE 8: note = MISC_FEATURE - Xaa is Ahp
  MOD_RES 14: note = METHYLATION
AVFVWNYXIIRRYYC

SEQ ID NO: 95 - protein, 15 aa, synthetic construct
  REGION 1..15: note = Synthesized polypeptide
  MOD_RES 3: note = METHYLATION
  SITE 8: note = MISC_FEATURE - Xaa is Ahp
  MOD_RES 14: note = METHYLATION
AVFVWNYXIIRRYYC

SEQ ID NO: 96 - protein, 15 aa, synthetic construct
  REGION 1..15: note = Synthesized polypeptide
  MOD_RES 3: note = METHYLATION
  MOD_RES 14: note = METHYLATION
AVFVWNYYIIRRYYC

SEQ ID NO: 97 - protein, 15 aa, synthetic construct
  REGION 1..15: note = Synthesized polypeptide
  MOD_RES 3: note = METHYLATION
  MOD_RES 14: note = METHYLATION
AVFVWNYYIIRRYYC

SEQ ID NO: 98 - protein, 15 aa, synthetic construct
  REGION 1..15: note = Synthesized polypeptide
  MOD_RES 3: note = METHYLATION
  MOD_RES 14: note = METHYLATION
AVFVWNYYIIRRYYC

SEQ ID NO: 99 - protein, 15 aa, synthetic construct
  REGION 1..15: note = Synthesized polypeptide
  MOD_RES 3: note = METHYLATION
  MOD_RES 14: note = METHYLATION
AVFVWNYYIIRRYYC

SEQ ID NO: 100 - protein, 15 aa, synthetic construct
  REGION 1..15: note = Synthesized polypeptide
  SITE 3: note = MISC_FEATURE - Xaa is MeF3C
  MOD_RES 5: note = METHYLATION
  SITE 8: note = MISC_FEATURE - Xaa is F4OMe
  SITE 12: note = MISC_FEATURE - Xaa is dr
  MOD_RES 14: note = METHYLATION
AVXVWNYXIIRXFYC

SEQ ID NO: 101 - protein, 15 aa, synthetic construct
  REGION 1..15: note = Synthesized polypeptide
  SITE 3: note = MISC_FEATURE - Xaa is MeF3C
  MOD_RES 5: note = METHYLATION
  SITE 8: note = MISC_FEATURE - Xaa is F4OMe
  SITE 12: note = MISC_FEATURE - Xaa is dr
  MOD_RES 14: note = METHYLATION
AVXVWNYXIIRXFYC

SEQ ID NO: 102 - protein, 15 aa, synthetic construct
  REGION 1..15: note = Synthesized polypeptide
  SITE 3: note = MISC_FEATURE - Xaa is MeF3C
  MOD_RES 5: note = METHYLATION
  SITE 8: note = MISC_FEATURE - Xaa is F4OMe
  SITE 12: note = MISC_FEATURE - Xaa is dr
  MOD_RES 14: note = METHYLATION
AVXVWNYXIIRXFYC

SEQ ID NO: 103 - protein, 15 aa, synthetic construct
  REGION 1..15: note = Synthesized polypeptide
  SITE 3: note = MISC_FEATURE - Xaa is MeF3C
  MOD_RES 5: note = METHYLATION
  SITE 8: note = MISC_FEATURE - Xaa is F4OMe
  SITE 12: note = MISC_FEATURE - Xaa is dr
  MOD_RES 14: note = METHYLATION
AVXVWNYXIIRXFYC

SEQ ID NO: 104 - protein, 15 aa, synthetic construct
  REGION 1..15: note = Synthesized polypeptide
AVFVWNYYIIRRFYC

SEQ ID NO: 105 - protein, 15 aa, synthetic construct
  REGION 1..15: note = Synthesized polypeptide
  SITE 3: note = MISC_FEATURE - Xaa is MeF3C
  SITE 8: note = MISC_FEATURE - Xaa is F4OMe
  SITE 12: note = MISC_FEATURE - Xaa is dr
  MOD_RES 14: note = METHYLATION
AVXVWNYXIIRXFYC

SEQ ID NO: 106 - protein, 15 aa, synthetic construct
  REGION 1..15: note = Synthesized polypeptide
  SITE 3: note = MISC_FEATURE - Xaa is MeF3C
  SITE 8: note = MISC_FEATURE - Xaa is F4OMe
  MOD_RES 14: note = METHYLATION
AVXVWNYXIIRRFYC

SEQ ID NO: 107 - protein, 15 aa, synthetic construct
  REGION 1..15: note = Synthesized polypeptide
  SITE 3: note = MISC_FEATURE - Xaa is MeF3C
  SITE 8: note = MISC_FEATURE - Xaa is F4OMe
  SITE 12: note = MISC_FEATURE - Xaa is dr
  MOD_RES 14: note = METHYLATION
AEXVWNYXIIRXFYC

SEQ ID NO: 108 - protein, 15 aa, synthetic construct
  REGION 1..15: note = Synthesized polypeptide
  MOD_RES 14: note = METHYLATION
AVFVWNYYIIRRYYC

SEQ ID NO: 109 - protein, 15 aa, synthetic construct
  REGION 1..15: note = Synthesized polypeptide
  MOD_RES 14: note = METHYLATION
AVFVWNYYIIRRYYC

SEQ ID NO: 110 - protein, 15 aa, synthetic construct
  REGION 1..15: note = Synthesized polypeptide
  MOD_RES 14: note = METHYLATION
AVFVWNYYIIRRYYC

SEQ ID NO: 111-130 - skipped (20 entries)

SEQ ID NO: 131 - protein, 6 aa, synthetic construct
  REGION 1..6: note = Synthesized polypeptide
  SITE 5: note = MISC_FEATURE - Xaa is PEG12
  SITE 6: note = MISC_FEATURE - Xaa is Hydrazide
GEGEXX

SEQ ID NO: 132 - skipped

SEQ ID NO: 133 - protein, 14 aa, synthetic construct
  REGION 1..14: note = Synthesized polypeptide
  SITE 13: note = MISC_FEATURE - Xaa is gAbu
  SITE 14: note = MISC_FEATURE - Xaa is NHS
GGGGSSGGGGSSXX

SEQ ID NO: 134 - protein, 14 aa, synthetic construct
  REGION 1..14: note = Synthesized polypeptide
  SITE 13: note = MISC_FEATURE - Xaa is gAbu
  SITE 14: note = MISC_FEATURE - Xaa is NHS
GGRGRSGGRGRSXX

SEQ ID NO: 135 - protein, 14 aa, synthetic construct
  REGION 1..14: note = Synthesized polypeptide
  SITE 13: note = MISC_FEATURE - Xaa is gAbu
  SITE 14: note = MISC_FEATURE - Xaa is NHS
GGQGQSGGQGQSXX

SEQ ID NO: 136 - protein, 13 aa, synthetic construct
  REGION 1..13: note = Synthesized polypeptide
  SITE 13: note = MISC_FEATURE - Xaa is K(Maleimide)
GGSGSSGGSGSSX

SEQ ID NO: 137 - protein, 10 aa, synthetic construct
  REGION 1..10: note = Synthesized polypeptide
  SITE 10: note = MISC_FEATURE - Xaa is K(Maleimide)
GGSGSSGSSX

SEQ ID NO: 138 - protein, 8 aa, synthetic construct
  REGION 1..8: note = Synthesized polypeptide
  SITE 7: note = MISC_FEATURE - Xaa is gAbu
  SITE 8: note = MISC_FEATURE - Xaa is NHS
GGQGQSXX

SEQ ID NO: 139 - protein, 8 aa, synthetic construct
  REGION 1..8: note = Synthesized polypeptide
  SITE 7: note = MISC_FEATURE - Xaa is gAbu
  SITE 8: note = MISC_FEATURE - Xaa is NHS
GGGGSSXX

SEQ ID NO: 140 - protein, 8 aa, synthetic construct
  REGION 1..8: note = Synthesized polypeptide
  SITE 7: note = MISC_FEATURE - Xaa is gAbu
  SITE 8: note = MISC_FEATURE - Xaa is NHS
GGRGRSXX

SEQ ID NO: 141 - protein, 7 aa, synthetic construct
  REGION 1..7: note = Synthesized polypeptide
  SITE 7: note = MISC_FEATURE - Xaa is KTrzMal
GGGGSSX

SEQ ID NO: 142 - protein, 7 aa, synthetic construct
  REGION 1..7: note = Synthesized polypeptide
  SITE 7: note = MISC_FEATURE - Xaa is K(Maleimide)
GSSGSSX

SEQ ID NO: 143 - protein, 7 aa, synthetic construct
  REGION 1..7: note = Synthesized polypeptide
  MOD_RES 2: note = METHYLATION
  MOD_RES 4: note = METHYLATION
  SITE 7: note = MISC_FEATURE - Xaa is K(Maleimide)
GGSGSSX

SEQ ID NO: 144 - protein, 7 aa, synthetic construct
  REGION 1..7: note = Synthesized polypeptide
  SITE 7: note = MISC_FEATURE - Xaa is K(Maleimide)
GGRGRSX

SEQ ID NO: 145 - protein, 7 aa, synthetic construct
  REGION 1..7: note = Synthesized polypeptide
  SITE 7: note = MISC_FEATURE - Xaa is K(Maleimide)
GGRSESX

SEQ ID NO: 146 - protein, 7 aa, synthetic construct
  REGION 1..7: note = Synthesized polypeptide
  SITE 7: note = MISC_FEATURE - Xaa is K(Maleimide)
GGGGSSX

SEQ ID NO: 147 - protein, 7 aa, synthetic construct
  REGION 1..7: note = Synthesized polypeptide
  SITE 7: note = MISC_FEATURE - Xaa is K(Maleimide)
GGSGSSX

SEQ ID NO: 148 - protein, 7 aa, synthetic construct
  REGION 1..7: note = Synthesized polypeptide
  SITE 7: note = MISC_FEATURE - Xaa is K(Maleimide)
GGSGESX

SEQ ID NO: 149 - protein, 7 aa, synthetic construct
  REGION 1..7: note = Synthesized polypeptide
  SITE 7: note = MISC_FEATURE - Xaa is K(Maleimide)
GGSGRSX

SEQ ID NO: 150 - protein, 7 aa, synthetic construct
  REGION 1..7: note = Synthesized polypeptide
  SITE 7: note = MISC_FEATURE - Xaa is K(Maleimide)
GGSGSGX

SEQ ID NO: 151 - protein, 7 aa, synthetic construct
  REGION 1..7: note = Synthesized polypeptide
  SITE 7: note = MISC_FEATURE - Xaa is dK(Maleimide)
GGSGSGX

SEQ ID NO: 152 - protein, 7 aa, synthetic construct
  REGION 1..7: note = Synthesized polypeptide
  SITE 7: note = MISC_FEATURE - Xaa is K(Maleimide)
GGESESX

SEQ ID NO: 153 - protein, 7 aa, synthetic construct
  REGION 1..7: note = Synthesized polypeptide
  SITE 3: note = MISC_FEATURE - Xaa is de
  SITE 5: note = MISC_FEATURE - Xaa is de
  SITE 7: note = MISC_FEATURE - Xaa is dK(Maleimide)
GGXGXGX

SEQ ID NO: 154 - protein, 12 aa, synthetic construct
  REGION 1..12: note = Synthesized polypeptide
  SITE 12: note = MISC_FEATURE - Xaa is dK(Maleimide)
GGSGSGGSSGGX

SEQ ID NO: 155 - protein, 12 aa, synthetic construct
  REGION 1..12: note = Synthesized polypeptide
  SITE 3: note = MISC_FEATURE - Xaa is de
  SITE 6: note = MISC_FEATURE - Xaa is de
  SITE 9: note = MISC_FEATURE - Xaa is de
  SITE 12: note = MISC_FEATURE - Xaa is dK(Maleimide)
GGXGGXGGXGGX

SEQ ID NO: 156 - protein, 6 aa, synthetic construct
  REGION 1..6: note = Synthesized polypeptide
  SITE 6: note = MISC_FEATURE - Xaa is K(Maleimide)
GGGSSX

SEQ ID NO: 157 - protein, 5 aa, synthetic construct
  REGION 1..5: note = Synthesized polypeptide
  SITE 5: note = MISC_FEATURE - Xaa is K(Maleimide)
GGSSX

SEQ ID NO: 158-161 - skipped (4 entries)